European Patent Specification EP 4 055 389 B1, published September 11, 2024. Title: DIAGNOSTICS AND USE OF QUORUM SENSING MOLECULES IN MUSCLE WASTING. Applicant: Universiteit Gent. The sequence listing filed with the application follows.

SEQUENCE LISTING (87 sequences)

SEQ ID NO: 1 - protein, 7 aa, AA-peptide
YSPWTNF

SEQ ID NO: 2 - protein, 7 aa, AA-peptide
ADLPFEF

SEQ ID NO: 3 - protein, 25 aa, AA-peptide
AGTKPQGKPASNLVECVFSLFKKCN

SEQ ID NO: 4 - protein, 7 aa, AA-peptide
AIFILAS

SEQ ID NO: 5 - protein, 7 aa, AA-peptide
AITLIFI

SEQ ID NO: 6 - protein, 5 aa, AA-peptide
AKDEH

SEQ ID NO: 7 - protein, 5 aa, AA-peptide
AKTVQ

SEQ ID NO: 8 - protein, 8 aa, AA-peptide
ALILTLVS

SEQ ID NO: 9 - protein, 5 aa, AA-peptide
ARNQT

SEQ ID NO: 10 - protein, 5 aa, AA-peptide
NNWNN

SEQ ID NO: 11 - protein, 5 aa, AA-peptide
CVGIW

SEQ ID NO: 12 - protein, 19 aa, AA-peptide
DIRHRINNSIWRDIFLKRK

SEQ ID NO: 13 - protein, 15 aa, AA-peptide
DLRGVPNPWGWIFGR

SEQ ID NO: 14 - protein, 14 aa, AA-peptide
DLRNIFLKIKFKKK

SEQ ID NO: 15 - protein, 5 aa, AA-peptide
DRVGA

SEQ ID NO: 16 - protein, 8 aa, AA-peptide
DSVCASYF

SEQ ID NO: 17 - protein, 17 aa, AA-peptide
DWRFLNSIRDLIFPKRK

SEQ ID NO: 18 - protein, 5 aa, AA-peptide
EKMIG

SEQ ID NO: 19 - protein, 17 aa, AA-peptide
EMRISRIILDFLFLRKK

SEQ ID NO: 20 - protein, 16 aa, AA-peptide
EMRKSNNNFFHFLRRI

SEQ ID NO: 21 - protein, 17 aa, AA-peptide
EMRLPKILRDFIFPRKK

SEQ ID NO: 22 - protein, 28 aa, AA-peptide
EQLSFTSIGILQLLTIGTRSCWFFYCRY

SEQ ID NO: 23 - protein, 5 aa, AA-peptide
ERGMT

SEQ ID NO: 24 - protein, 5 aa, AA-peptide
ERNNT

SEQ ID NO: 25 - protein, 5 aa, AA-peptide
ERPVG

SEQ ID NO: 26 - protein, 17 aa, AA-peptide
ESRLPKILLDFLFLRKK

SEQ ID NO: 27 - protein, 17 aa, AA-peptide
ESRLPKIRFDFIFPRKK

SEQ ID NO: 28 - protein, 17 aa, AA-peptide
ESRVSRIILDFLFQRKK

SEQ ID NO: 29 - protein, 25 aa, AA-peptide
VNYGNGVSCSKTKCSVNWGQAFQER

SEQ ID NO: 30 - protein, 16 aa, AA-peptide
DSRIRMGFDFSKLFGK

SEQ ID NO: 31 - protein, 17 aa, AA-peptide
ESRISDILLDFLFQRKK

SEQ ID NO: 32 - protein, 12 aa, AA-peptide
FHWWQTSPAHFS

SEQ ID NO: 33 - protein, 8 aa, AA-peptide
FLVMFLSG

SEQ ID NO: 34 - protein, 11 aa, AA-peptide
QNSPNIFGQWM

SEQ ID NO: 35 - protein, 5 aa, AA-peptide
GKAEF

SEQ ID NO: 36 - protein, 27 aa, AA-peptide
GLWEDILYSLNIIKHNNTKGLHHPIQL

SEQ ID NO: 37 - protein, 18 aa, AA-peptide
GLWEDLLYNINRYAHYIT

SEQ ID NO: 38 - protein, 10 aa, AA-peptide
ILSGAPCIPW

SEQ ID NO: 39 - protein, 5 aa, AA-peptide
IRFVT

SEQ ID NO: 40 - protein, 26 aa, AA-peptide
KSSAYSLQMGATAIKQVKKLFKKWGW

SEQ ID NO: 41 - protein, 9 aa, AA-peptide
KYYPCFGYF

SEQ ID NO: 42 - protein, 8 aa, AA-peptide
LFSLVLAG

SEQ ID NO: 43 - protein, 8 aa, AA-peptide
LFVVTLVG

SEQ ID NO: 44 - protein, 5 aa, AA-peptide
LPFEF

SEQ ID NO: 45 - protein, 5 aa, AA-peptide
LPFEH

SEQ ID NO: 46 - protein, 6 aa, AA-peptide
LVTLVF

SEQ ID NO: 47 - protein, 19 aa, AA-peptide
MAGNSSNFIHKIKQIFTHR

SEQ ID NO: 48 - protein, 5 aa, AA-peptide
MKAEH

SEQ ID NO: 49 - protein, 5 aa, AA-peptide
MPFEF

SEQ ID NO: 50 - protein, 7 aa, AA-peptide
NEVPFEF

SEQ ID NO: 51 - protein, 8 aa, AA-peptide
YSTCDFIM

SEQ ID NO: 52 - protein, 5 aa, AA-peptide
QKGMY

SEQ ID NO: 53 - protein, 5 aa, AA-peptide
QRGMI

SEQ ID NO: 54 - protein, 7 aa, AA-peptide
SDLPFEH

SEQ ID NO: 55 - protein, 7 aa, AA-peptide
SDMPFEF

SEQ ID NO: 56 - protein, 21 aa, AA-peptide
SGSLSTFFRLFNRSFTQALGK

SEQ ID NO: 57 - protein, 7 aa, AA-peptide
SIFTLVA

SEQ ID NO: 58 - protein, 5 aa, AA-peptide
SKDYN

SEQ ID NO: 59 - protein, 5 aa, AA-peptide
SRKAT

SEQ ID NO: 60 - protein, 5 aa, AA-peptide
SRNAT

SEQ ID NO: 61 - protein, 5 aa, AA-peptide
SRNVT

SEQ ID NO: 62 - protein, 7 aa, AA-peptide
SYPGWSW

SEQ ID NO: 63 - protein, 23 aa, AA-peptide
TNRNYGKPNKDIGTCIWSGFRHC

SEQ ID NO: 64 - protein, 8 aa, AA-peptide
VAVLVLGA

SEQ ID NO: 65 - protein, 5 aa, AA-peptide
VPFEF

SEQ ID NO: 66 - protein, 12 aa, AA-peptide
WPFAHWPWQYPR

SEQ ID NO: 67 - protein, 8 aa, AA-peptide
YNPCSNYL

SEQ ID NO: 68 - protein, 7 aa, AA-peptide
ILIIVGG

SEQ ID NO: 69 - DNA, 20 bp, Artificial sequence
  primer
tgaatagcatccagatcagc

SEQ ID NO: 70 - DNA, 20 bp, Artificial sequence
  primer
cctctctgagaagtggtact

SEQ ID NO: 71 - DNA, 20 bp, Artificial sequence
  primer
aagactgagctgagtaactg

SEQ ID NO: 72 - DNA, 20 bp, Artificial sequence
  primer
gtagagggtgtcaaacttct

SEQ ID NO: 73 - DNA, 21 bp, Artificial sequence
  primer
tgtatgcttactctacagcac

SEQ ID NO: 74 - DNA, 19 bp, Artificial sequence
  primer
aaggactcgaattccgttg

SEQ ID NO: 75 - DNA, 20 bp, Artificial sequence
  primer
catcttcctgctaatggaca

SEQ ID NO: 76 - DNA, 20 bp, Artificial sequence
  primer
aaaggtatcaaaccccaagg

SEQ ID NO: 77 - protein, 16 aa, Artificial sequence
  Amino acid
SRVSAIILDFLFQRKK

SEQ ID NO: 78 - protein, 17 aa, Artificial sequence
  Amino acid
ESRVSRIIADFLFQRKK

SEQ ID NO: 79 - protein, 20 aa, Artificial sequence
  Amino acid
GSLSTFFALFNRSFTQALGK

SEQ ID NO: 80 - protein, 20 aa, Artificial sequence
  Amino acid
GSLSTFFRLFNASFTQALGK

SEQ ID NO: 81 - DNA, 15 bp, Artificial sequence
  Nucleotide sequence
tgtgtaggaatttgg

SEQ ID NO: 82 - DNA, 51 bp, Artificial sequence
  Nucleotide sequence
gaaagtagactgccaaaaatccgatttgattttattttcccacgaaaaaag

SEQ ID NO: 83 - DNA, 51 bp, Artificial sequence
  Nucleotide sequence
gaaagtagggtttcaagaatcatccttgattttcttttccaacgaaaaaag

SEQ ID NO: 84 - DNA, 78 bp, Artificial sequence
  Nucleotide sequence
aagagtagtgcgtattctttgcagatgggggcaactgcaattaaacaggtaaagaaactgtttaaaaaatggggatgg

SEQ ID NO: 85 - DNA, 66 bp, Artificial sequence
  Nucleotide sequence
agcggaagcctatcaacatttttccggctgtttaacagaagttttacacaagctttgggaaaataa

SEQ ID NO: 86 - DNA, 21 bp, Artificial sequence
  Nucleotide sequence
agtatttttactttagtagca

SEQ ID NO: 87 - DNA, 18 bp, Artificial sequence
  Nucleotide sequence
tcaaggaatgcaacatga